European Patent Specification EP 3 942 068 B1, published February 26, 2025. Title: METHODS AND SYSTEMS FOR DETECTING METHYLATION CHANGES IN DNA SAMPLES. Applicant: NUCLEIX LTD. The sequence listing filed with the application follows.

SEQUENCE LISTING (11 sequences)

SEQ ID NO: 1 - DNA, 85 bp, Homo sapiens
agtagcgcccactgagcggtttttcagttgctgcaccgttcttagcgcccaacggaacgtttcccgtacgcggagtccataagtt

SEQ ID NO: 2 - DNA, 69 bp, Homo sapiens
cggtcccgcagcgcccgccacacacccgcgccagaggtccagcgcatgtgcagtgaaatggcctagccc

SEQ ID NO: 3 - DNA, 72 bp, Homo sapiens
cggatagcgcggcgggcgacagccccccggataaccccgccgagggaggggcgcttgtaaaaccgagcggcg

SEQ ID NO: 4 - DNA, 60 bp, Homo sapiens
tcctccttgccttctttcgccgaaagggggcgcgctcctcccaggctgcgctggtaccta

SEQ ID NO: 5 - DNA, 78 bp, Homo sapiens
aggacccgctccgcaaagcgcccaccctcgagggaggaaagccgagctgcgcctccgcgcaaggccagggagtgtggc

SEQ ID NO: 6 - DNA, 73 bp, Homo sapiens
aggccgcgagcgcggcgcgatcagtagcgcccactaacagttcgttctgcacggcggagcgcgagaccgcgga

SEQ ID NO: 7 - DNA, 60 bp, Homo sapiens
agactaacttttctcttgtacagaatcatcaggctaaatttttggcattatttcagtcct

SEQ ID NO: 8 - DNA, 33 bp, Artificial Sequence
  Oligonucleotide
tcgtcggcagcgtcagatgtgtataagagacag

SEQ ID NO: 9 - DNA, 34 bp, Artificial Sequence
  Oligonucleotide
gtctcgtgggctcggagatgtgtataagagacag

SEQ ID NO: 10 - DNA, 24 bp, Artificial Sequence
  Primer
ttaaaacaagatttacctctattg

SEQ ID NO: 11 - DNA, 24 bp, Artificial Sequence
  Primer
aaatgactgaatataaacttgtgg